European Patent Specification EP 3 997 219 B1, published August 6, 2025. Title: NOVEL ESTERASES AND USES THEREOF. Applicant: CARBIOS. The sequence listing filed with the application follows.

SEQUENCE LISTING (2 sequences)

SEQ ID NO: 1 - protein, 264 aa, Ideonella sakaiensis
MQTNPYARGPNPTAASLEASAGPFTVRSFTVSRPSGYGAGTVYYPTNAGGTVGAIAIVPGYTARQSSIKWWGPRLASHGFVVITIDTNSTLDQPSSRSSQQMAALRQVASLNGTSSSPIYGKVDTARMGVMGWSMGGGGSLISAANNPSLKAAAPQAPWDSSTNFSSVTVPTLIFACENDSIAPVNSSALPIYDSMSRNAKQFLEINGGSHSCANSGNSNQALIGKKGVAWMKRFMDNDTRYSTFACENPNSTRVSDFRTANCS

SEQ ID NO: 2 - protein, 21 aa, artificial sequence
  PelB leader sequence
KYLLPTAAAGLLLLAAQPAMA